European Patent Specification EP 3 689 900 B1, published July 23, 2025. Title: ANTI-HUMAN PAPILLOMAVIRUS 16 E7 T CELL RECEPTORS. Applicant: THE UNITED STATES OF AMERICA, AS REPRESENTED BY THE SECRETARY, DEPARTMENT OF HEALTH AND HUMAN SERVICES. Application EP. The sequence listing filed with the application follows.

SEQUENCE LISTING (40 sequences)

SEQ ID NO: 1 - protein, 98 aa, Artificial Sequence
  Synthetic
MHGDTPTLHEYMLDLQPETTDLYCYEQLNDSSEEEDEIDGPAGQAEPDRAHYNIVTFCCKCDSTLRLCVQSTHVDIRTLEDLLMGTLGIVCPICSQKP

SEQ ID NO: 2 - protein, 9 aa, Artificial Sequence
  Synthetic
YMLDLQPET

SEQ ID NO: 3 - protein, 6 aa, Artificial Sequence
  Synthetic
TSGFNG

SEQ ID NO: 4 - protein, 6 aa, Artificial Sequence
  Synthetic
NVLDGL

SEQ ID NO: 5 - protein, 10 aa, Artificial Sequence
  Synthetic
ASVDGNNRLA

SEQ ID NO: 6 - protein, 5 aa, Artificial Sequence
  Synthetic
SGHDT

SEQ ID NO: 7 - protein, 6 aa, Artificial Sequence
  Synthetic
YYEEEE

SEQ ID NO: 8 - protein, 15 aa, Artificial Sequence
  Synthetic
ASSLGWRGGRYNEQF

SEQ ID NO: 9 - protein, 126 aa, Artificial Sequence
  Synthetic
MWGVFLLYVSMKMGGTTGQNIDQPTEMTATEGAIVQINCTYQTSGFNGLFWYQQHAGEAPTFLSYNVLDGLEEKGRFSSFLSRSKGYSYLLLKELQMKDSASYLCASVDGNNRLAFGKGNQVVVIP

SEQ ID NO: 10 - protein, 135 aa, Artificial Sequence
  Synthetic
  MISC_FEATURE (2)..(2): Xaa is Ala or Gly
MXPGLLCWALLCLLGAGLVDAGVTQSPTHLIKTRGQQVTLRCSPKSGHDTVSWYQQALGQGPQFIFQYYEEEERQRGNFPDRFSGHQFPNYSSELNVNALLLGDSALYLCASSLGWRGGRYNEQFFGPGTRLTVL

SEQ ID NO: 11 - protein, 135 aa, Artificial Sequence
  Synthetic
MGPGLLCWALLCLLGAGLVDAGVTQSPTHLIKTRGQQVTLRCSPKSGHDTVSWYQQALGQGPQFIFQYYEEEERQRGNFPDRFSGHQFPNYSSELNVNALLLGDSALYLCASSLGWRGGRYNEQFFGPGTRLTVL

SEQ ID NO: 12 - protein, 267 aa, Artificial Sequence
  Synthetic
MWGVFLLYVSMKMGGTTGQNIDQPTEMTATEGAIVQINCTYQTSGFNGLFWYQQHAGEAPTFLSYNVLDGLEEKGRFSSFLSRSKGYSYLLLKELQMKDSASYLCASVDGNNRLAFGKGNQVVVIPNIQNPDPAVYQLRDSKSSDKSVCLFTDFDSQTNVSQSKDSDVYITDKTVLDMRSMDFKSNSAVAWSNKSDFACANAFNNSIIPEDTFFPSPESSCDVKLVEKSFETDTNLNFQNLSVIGFRILLLKVAGFNLLMTLRLWSS

SEQ ID NO: 13 - protein, 314 aa, Artificial Sequence
  Synthetic
MGPGLLCWALLCLLGAGLVDAGVTQSPTHLIKTRGQQVTLRCSPKSGHDTVSWYQQALGQGPQFIFQYYEEEERQRGNFPDRFSGHQFPNYSSELNVNALLLGDSALYLCASSLGWRGGRYNEQFFGPGTRLTVLEDLKNVFPPEVAVFEPSEAEISHTQKATLVCLATGFYPDHVELSWWVNGKEVHSGVSTDPQPLKEQPALNDSRYCLSSRLRVSATFWQNPRNHFRCQVQFYGLSENDEWTQDRAKPVTQIVSAEAWGRADCGFTSESYQQGVLSATILYEILLGKATLYAVLVSALVLMAMVKRKDSRG

SEQ ID NO: 14 - protein, 141 aa, Artificial Sequence
  Synthetic
NIQNPDPAVYQLRDSKSSDKSVCLFTDFDSQTNVSQSKDSDVYITDKTVLDMRSMDFKSNSAVAWSNKSDFACANAFNNSIIPEDTFFPSPESSCDVKLVEKSFETDTNLNFQNLSVIGFRILLLKVAGFNLLMTLRLWSS

SEQ ID NO: 15 - protein, 179 aa, Artificial Sequence
  Synthetic
EDLKNVFPPEVAVFEPSEAEISHTQKATLVCLATGFYPDHVELSWWVNGKEVHSGVSTDPQPLKEQPALNDSRYCLSSRLRVSATFWQNPRNHFRCQVQFYGLSENDEWTQDRAKPVTQIVSAEAWGRADCGFTSESYQQGVLSATILYEILLGKATLYAVLVSALVLMAMVKRKDSRG

SEQ ID NO: 16 - protein, 137 aa, Artificial Sequence
  Synthetic
  MISC_FEATURE (48)..(48): Xaa is Thr or Cys
  MISC_FEATURE (112)..(112): Xaa is Ser, Gly, Ala, Val, Leu, Ile, Pro, Phe, Met, or Trp
  MISC_FEATURE (114)..(114): Xaa is Met, Gly, Ala, Val, Leu, Ile, Pro, Phe, Met, or Trp
  MISC_FEATURE (115)..(115): Xaa is Gly, Ala, Val, Leu, Ile, Pro, Phe, Met, or Trp
NIQNPEPAVYQLKDPRSQDSTLCLFTDFDSQINVPKTMESGTFITDKXVLDMKAMDSKSNGAIAWSNQTSFTCQDIFKETNATYPSSDVPCDATLTEKSFETDMNLNFQNLXVXXLRILLLKVAGFNLLMTLRLWSS

SEQ ID NO: 17 - protein, 137 aa, Artificial Sequence
  Synthetic
NIQNPEPAVYQLKDPRSQDSTLCLFTDFDSQINVPKTMESGTFITDKTVLDMKAMDSKSNGAIAWSNQTSFTCQDIFKETNATYPSSDVPCDATLTEKSFETDMNLNFQNLSVMGLRILLLKVAGFNLLMTLRLWSS

SEQ ID NO: 18 - protein, 173 aa, Artificial Sequence
  Synthetic
  MISC_FEATURE (57)..(57): Xaa is Ser or Cys
EDLRNVTPPKVSLFEPSKAEIANKQKATLVCLARGFFPDHVELSWWVNGKEVHSGVXTDPQAYKESNYSYCLSSRLRVSATFWHNPRNHFRCQVQFHGLSEEDKWPEGSPKPVTQNISAEAWGRADCGITSASYQQGVLSATILYEILLGKATLYAVLVSTLVVMAMVKRKNS

SEQ ID NO: 19 - protein, 173 aa, Artificial Sequence
  Synthetic
EDLRNVTPPKVSLFEPSKAEIANKQKATLVCLARGFFPDHVELSWWVNGKEVHSGVSTDPQAYKESNYSYCLSSRLRVSATFWHNPRNHFRCQVQFHGLSEEDKWPEGSPKPVTQNISAEAWGRADCGITSASYQQGVLSATILYEILLGKATLYAVLVSTLVVMAMVKRKNS

SEQ ID NO: 20 - protein, 308 aa, Artificial Sequence
  Synthetic
MAPGLLCWALLCLLGAGLVDAGVTQSPTHLIKTRGQQVTLRCSPKSGHDTVSWYQQALGQGPQFIFQYYEEEERQRGNFPDRFSGHQFPNYSSELNVNALLLGDSALYLCASSLGWRGGRYNEQFFGPGTRLTVLEDLRNVTPPKVSLFEPSKAEIANKQKATLVCLARGFFPDHVELSWWVNGKEVHSGVSTDPQAYKESNYSYCLSSRLRVSATFWHNPRNHFRCQVQFHGLSEEDKWPEGSPKPVTQNISAEAWGRADCGITSASYQQGVLSATILYEILLGKATLYAVLVSTLVVMAMVKRKNS

SEQ ID NO: 21 - protein, 137 aa, Artificial Sequence
  Synthetic
NIQNPEPAVYQLKDPRSQDSTLCLFTDFDSQINVPKTMESGTFITDKTVLDMKAMDSKSNGAIAWSNQTSFTCQDIFKETNATYPSSDVPCDATLTEKSFETDMNLNFQNLLVIVLRILLLKVAGFNLLMTLRLWSS

SEQ ID NO: 22 - protein, 263 aa, Artificial Sequence
  Synthetic
MWGVFLLYVSMKMGGTTGQNIDQPTEMTATEGAIVQINCTYQTSGFNGLFWYQQHAGEAPTFLSYNVLDGLEEKGRFSSFLSRSKGYSYLLLKELQMKDSASYLCASVDGNNRLAFGKGNQVVVIPNIQNPEPAVYQLKDPRSQDSTLCLFTDFDSQINVPKTMESGTFITDKTVLDMKAMDSKSNGAIAWSNQTSFTCQDIFKETNATYPSSDVPCDATLTEKSFETDMNLNFQNLLVIVLRILLLKVAGFNLLMTLRLWSS

SEQ ID NO: 23 - protein, 173 aa, Artificial Sequence
  Synthetic
EDLRNVTPPKVSLFEPSKAEIANKQKATLVCLARGFFPDHVELSWWVNGKEVHSGVCTDPQAYKESNYSYCLSSRLRVSATFWHNPRNHFRCQVQFHGLSEEDKWPEGSPKPVTQNISAEAWGRADCGITSASYQQGVLSATILYEILLGKATLYAVLVSTLVVMAMVKRKNS

SEQ ID NO: 24 - protein, 137 aa, Artificial Sequence
  Synthetic
NIQNPEPAVYQLKDPRSQDSTLCLFTDFDSQINVPKTMESGTFITDKCVLDMKAMDSKSNGAIAWSNQTSFTCQDIFKETNATYPSSDVPCDATLTEKSFETDMNLNFQNLSVMGLRILLLKVAGFNLLMTLRLWSS

SEQ ID NO: 25 - protein, 137 aa, Artificial Sequence
  Synthetic
NIQNPEPAVYQLKDPRSQDSTLCLFTDFDSQINVPKTMESGTFITDKCVLDMKAMDSKSNGAIAWSNQTSFTCQDIFKETNATYPSSDVPCDATLTEKSFETDMNLNFQNLLVIVLRILLLKVAGFNLLMTLRLWSS

SEQ ID NO: 26 - protein, 263 aa, Artificial Sequence
  Synthetic
MWGVFLLYVSMKMGGTTGQNIDQPTEMTATEGAIVQINCTYQTSGFNGLFWYQQHAGEAPTFLSYNVLDGLEEKGRFSSFLSRSKGYSYLLLKELQMKDSASYLCASVDGNNRLAFGKGNQVVVIPNIQNPEPAVYQLKDPRSQDSTLCLFTDFDSQINVPKTMESGTFITDKCVLDMKAMDSKSNGAIAWSNQTSFTCQDIFKETNATYPSSDVPCDATLTEKSFETDMNLNFQNLLVIVLRILLLKVAGFNLLMTLRLWSS

SEQ ID NO: 27 - protein, 308 aa, Artificial Sequence
  Synthetic
MAPGLLCWALLCLLGAGLVDAGVTQSPTHLIKTRGQQVTLRCSPKSGHDTVSWYQQALGQGPQFIFQYYEEEERQRGNFPDRFSGHQFPNYSSELNVNALLLGDSALYLCASSLGWRGGRYNEQFFGPGTRLTVLEDLRNVTPPKVSLFEPSKAEIANKQKATLVCLARGFFPDHVELSWWVNGKEVHSGVCTDPQAYKESNYSYCLSSRLRVSATFWHNPRNHFRCQVQFHGLSEEDKWPEGSPKPVTQNISAEAWGRADCGITSASYQQGVLSATILYEILLGKATLYAVLVSTLVVMAMVKRKNS

SEQ ID NO: 28 - protein, 27 aa, Artificial Sequence
  Synthetic
RAKRSGSGATNFSLLKQAGDVEENPGP

SEQ ID NO: 29 - protein, 598 aa, Artificial Sequence
  Synthetic
MAPGLLCWALLCLLGAGLVDAGVTQSPTHLIKTRGQQVTLRCSPKSGHDTVSWYQQALGQGPQFIFQYYEEEERQRGNFPDRFSGHQFPNYSSELNVNALLLGDSALYLCASSLGWRGGRYNEQFFGPGTRLTVLEDLRNVTPPKVSLFEPSKAEIANKQKATLVCLARGFFPDHVELSWWVNGKEVHSGVSTDPQAYKESNYSYCLSSRLRVSATFWHNPRNHFRCQVQFHGLSEEDKWPEGSPKPVTQNISAEAWGRADCGITSASYQQGVLSATILYEILLGKATLYAVLVSTLVVMAMVKRKNSRAKRSGSGATNFSLLKQAGDVEENPGPMWGVFLLYVSMKMGGTTGQNIDQPTEMTATEGAIVQINCTYQTSGFNGLFWYQQHAGEAPTFLSYNVLDGLEEKGRFSSFLSRSKGYSYLLLKELQMKDSASYLCASVDGNNRLAFGKGNQVVVIPNIQNPEPAVYQLKDPRSQDSTLCLFTDFDSQINVPKTMESGTFITDKTVLDMKAMDSKSNGAIAWSNQTSFTCQDIFKETNATYPSSDVPCDATLTEKSFETDMNLNFQNLLVIVLRILLLKVAGFNLLMTLRLWSS

SEQ ID NO: 30 - protein, 598 aa, Artificial Sequence
  Synthetic
MAPGLLCWALLCLLGAGLVDAGVTQSPTHLIKTRGQQVTLRCSPKSGHDTVSWYQQALGQGPQFIFQYYEEEERQRGNFPDRFSGHQFPNYSSELNVNALLLGDSALYLCASSLGWRGGRYNEQFFGPGTRLTVLEDLRNVTPPKVSLFEPSKAEIANKQKATLVCLARGFFPDHVELSWWVNGKEVHSGVCTDPQAYKESNYSYCLSSRLRVSATFWHNPRNHFRCQVQFHGLSEEDKWPEGSPKPVTQNISAEAWGRADCGITSASYQQGVLSATILYEILLGKATLYAVLVSTLVVMAMVKRKNSRAKRSGSGATNFSLLKQAGDVEENPGPMWGVFLLYVSMKMGGTTGQNIDQPTEMTATEGAIVQINCTYQTSGFNGLFWYQQHAGEAPTFLSYNVLDGLEEKGRFSSFLSRSKGYSYLLLKELQMKDSASYLCASVDGNNRLAFGKGNQVVVIPNIQNPEPAVYQLKDPRSQDSTLCLFTDFDSQINVPKTMESGTFITDKCVLDMKAMDSKSNGAIAWSNQTSFTCQDIFKETNATYPSSDVPCDATLTEKSFETDMNLNFQNLLVIVLRILLLKVAGFNLLMTLRLWSS

SEQ ID NO: 31 - DNA, 804 bp, Artificial Sequence
  Synthetic
atgtggggagttttccttctttatgtttccatgaagatgggaggcactacaggacaaaacattgaccagcccactgagatgacagctacggaaggtgccattgtccagatcaactgcacgtaccagacatctgggttcaacgggctgttctggtaccagcaacatgctggcgaagcacccacatttctgtcttacaatgttctggatggtttggaggagaaaggtcgtttttcttcattccttagtcggtctaaagggtacagttacctccttttgaaggagctccagatgaaagactctgcctcttacctctgtgcttccgtagatgggaacaacagactcgcttttgggaaggggaaccaagtggtggtcataccaaatatccagaaccctgaccctgccgtgtaccagctgagagactctaaatccagtgacaagtctgtctgcctattcaccgattttgattctcaaacaaatgtgtcacaaagtaaggattctgatgtgtatatcacagacaaaactgtgctagacatgaggtctatggacttcaagagcaacagtgctgtggcctggagcaacaaatctgactttgcatgtgcaaacgccttcaacaacagcattattccagaagacaccttcttccccagcccagaaagttcctgtgatgtcaagctggtcgagaaaagctttgaaacagatacgaacctaaactttcaaaacctgtcagtgattgggttccgaatcctcctcctgaaagtggccgggtttaatctgctcatgacgctgcggctgtggtccagctga

SEQ ID NO: 32 - DNA, 945 bp, Artificial Sequence
  Synthetic
atgggccccgggctcctctgctgggcactgctttgtctcctgggagcaggcttagtggacgctggagtcacccaaagtcccacacacctgatcaaaacgagaggacagcaagtgactctgagatgctctcctaagtctgggcatgacactgtgtcctggtaccaacaggccctgggtcaggggccccagtttatctttcagtattatgaggaggaagagagacagagaggcaacttccctgatcgattctcaggtcaccagttccctaactatagctctgagctgaatgtgaacgccttgttgctgggggactcggccctctatctctgtgccagcagcttgggatggcgggggggccgttacaatgagcagttcttcgggccagggacacggctcaccgtgctagaggacctgaaaaacgtgttcccacccgaggtcgctgtgtttgagccatcagaagcagagatctcccacacccaaaaggccacactggtgtgcctggccacaggcttctaccccgaccacgtggagctgagctggtgggtgaatgggaaggaggtgcacagtggggtcagcacagacccgcagcccctcaaggagcagcccgccctcaatgactccagatactgcctgagcagccgcctgagggtctcggccaccttctggcagaacccccgcaaccacttccgctgtcaagtccagttctacgggctctcggagaatgacgagtggacccaggatagggccaaacctgtcacccagatcgtcagcgccgaggcctggggtagagcagactgtggcttcacctccgagtcttaccagcaaggggtcctgtctgccaccatcctctatgagatcttgctagggaaggccaccttgtatgccgtgctggtcagtgccctcgtgctgatggccatggtcaagagaaaggattccagaggctag

SEQ ID NO: 33 - DNA, 795 bp, Artificial Sequence
  Synthetic
atgtggggtgtcttccttttgtacgtcagcatgaagatgggaggcactactgggcaaaacatagatcagcctaccgaaatgactgctaccgagggagccattgtccaaatcaactgcacctatcagactagcggcttcaatggactcttctggtaccaacagcatgcgggcgaagcacctaccttcttgtcctataatgtcttggatggtctcgaagagaaaggcagattctccagtttcctcagccggagcaagggatactcatatcttctcctgaaagagcttcagatgaaggattctgcatcctatctctgtgcttcagtcgatggcaataaccgactcgcctttggaaaagggaatcaagtggtcgtcataccgaatattcagaaccccgaaccagccgtatatcagttgaaggacccaagatctcaggatagtacactctgtttgtttacggactttgactcacaaatcaacgtcccgaagactatggaaagtggtacgttcatcacagataagacggttctggacatgaaggctatggactcaaagagcaacggggcaattgcttggtccaaccagacaagctttacctgtcaggacatttttaaggagactaatgctacttatccctccagcgacgttccgtgtgatgcgactcttaccgagaagtcttttgagaccgatatgaatctcaacttccagaatctgctggtgatcgttctgcggatcctgcttctgaaggttgcaggattcaatcttcttatgactctccggctctggtcttcatgataa

SEQ ID NO: 34 - DNA, 924 bp, Artificial Sequence
  Synthetic
atggccccggggcttttgtgttgggccttgctttgtttgcttggggcaggcttggtggatgctggagtcacacagtcacccacacacctcattaaaaccaggggacaacaagtcactctgcgctgcagtcctaagtcaggccatgacacagtttcctggtatcaacaggctctggggcagggccctcagttcattttccaatattacgaggaagaggaacgccaacgcggtaatttccccgatcggttctctgggcaccagttcccaaactactcaagtgagttgaacgtaaatgctctcctcctcggagactccgccctctacttgtgtgccagttctcttggttggcggggcggccgatacaatgaacaattttttggacctggtactcggctgaccgtgctagaggacctgcgcaacgtcaccccaccaaaggtcagtttgtttgagccatcaaaggcggagatcgccaacaaacagaaagctacgctcgtgtgtttggctcggggcttcttcccagaccacgtagaactttcctggtgggtcaatggaaaggaggttcattccggagtgtccactgatccccaagcgtacaaggaatccaactatagctactgtctctcatctcggctccgggtgagtgcgacattctggcataatcctcggaaccactttcgatgccaagtgcagtttcatgggttgagcgaggaagacaagtggcccgagggcagtcctaaaccagtcactcaaaacataagcgccgaggcatggggtagagccgattgtgggattactagcgcttcataccaacaaggggtattgagcgctacaattctttacgaaattctcctcggcaaggcgacgctctacgccgtactggtgtctactctcgtggttatggcaatggtgaaacggaaaaacagc

SEQ ID NO: 35 - DNA, 795 bp, Artificial Sequence
  Synthetic
atgtggggtgtcttccttttgtacgtcagcatgaagatgggaggcactactgggcaaaacatagatcagcctaccgaaatgactgctaccgagggagccattgtccaaatcaactgcacctatcagactagcggcttcaatggactcttctggtaccaacagcatgcgggcgaagcacctaccttcttgtcctataatgtcttggatggtctcgaagagaaaggcagattctccagtttcctcagccggagcaagggatactcatatcttctcctgaaagagcttcagatgaaggattctgcatcctatctctgtgcttcagtcgatggcaataaccgactcgcctttggaaaagggaatcaagtggtcgtcataccgaatattcagaaccccgaaccagccgtatatcagttgaaggacccaagatctcaggatagtacactctgtttgtttacggactttgactcacaaatcaacgtcccgaagactatggaaagtggtacgttcatcacagataagtgcgttctggacatgaaggctatggactcaaagagcaacggggcaattgcttggtccaaccagacaagctttacctgtcaggacatttttaaggagactaatgctacttatccctccagcgacgttccgtgtgatgcgactcttaccgagaagtcttttgagaccgatatgaatctcaacttccagaatctgctggtgatcgttctgcggatcctgcttctgaaggttgcaggattcaatcttcttatgactctccggctctggtcttcatgataa

SEQ ID NO: 36 - DNA, 924 bp, Artificial Sequence
  Synthetic
atggccccggggcttttgtgttgggccttgctttgtttgcttggggcaggcttggtggatgctggagtcacacagtcacccacacacctcattaaaaccaggggacaacaagtcactctgcgctgcagtcctaagtcaggccatgacacagtttcctggtatcaacaggctctggggcagggccctcagttcattttccaatattacgaggaagaggaacgccaacgcggtaatttccccgatcggttctctgggcaccagttcccaaactactcaagtgagttgaacgtaaatgctctcctcctcggagactccgccctctacttgtgtgccagttctcttggttggcggggcggccgatacaatgaacaattttttggacctggtactcggctgaccgtgctagaggacctgcgcaacgtcaccccaccaaaggtcagtttgtttgagccatcaaaggcggagatcgccaacaaacagaaagctacgctcgtgtgtttggctcggggcttcttcccagaccacgtagaactttcctggtgggtcaatggaaaggaggttcattccggagtgtgcactgatccccaagcgtacaaggaatccaactatagctactgtctctcatctcggctccgggtgagtgcgacattctggcataatcctcggaaccactttcgatgccaagtgcagtttcatgggttgagcgaggaagacaagtggcccgagggcagtcctaaaccagtcactcaaaacataagcgccgaggcatggggtagagccgattgtgggattactagcgcttcataccaacaaggggtattgagcgctacaattctttacgaaattctcctcggcaaggcgacgctctacgccgtactggtgtctactctcgtggttatggcaatggtgaaacggaaaaacagc

SEQ ID NO: 37 - DNA, 7310 bp, Artificial Sequence
  Synthetic
ccatggccccggggcttttgtgttgggccttgctttgtttgcttggggcaggcttggtggatgctggagtcacacagtcacccacacacctcattaaaaccaggggacaacaagtcactctgcgctgcagtcctaagtcaggccatgacacagtttcctggtatcaacaggctctggggcagggccctcagttcattttccaatattacgaggaagaggaacgccaacgcggtaatttccccgatcggttctctgggcaccagttcccaaactactcaagtgagttgaacgtaaatgctctcctcctcggagactccgccctctacttgtgtgccagttctcttggttggcggggcggccgatacaatgaacaattttttggacctggtactcggctgaccgtgctagaggacctgcgcaacgtcaccccaccaaaggtcagtttgtttgagccatcaaaggcggagatcgccaacaaacagaaagctacgctcgtgtgtttggctcggggcttcttcccagaccacgtagaactttcctggtgggtcaatggaaaggaggttcattccggagtgtccactgatccccaagcgtacaaggaatccaactatagctactgtctctcatctcggctccgggtgagtgcgacattctggcataatcctcggaaccactttcgatgccaagtgcagtttcatgggttgagcgaggaagacaagtggcccgagggcagtcctaaaccagtcactcaaaacataagcgccgaggcatggggtagagccgattgtgggattactagcgcttcataccaacaaggggtattgagcgctacaattctttacgaaattctcctcggcaaggcgacgctctacgccgtactggtgtctactctcgtggttatggcaatggtgaaacggaaaaacagcagagccaaaagaagtggttctggcgcgacgaattttagtttgcttaagcaagccggagatgtggaggaaaatcctggaccgatgtggggtgtcttccttttgtacgtcagcatgaagatgggaggcactactgggcaaaacatagatcagcctaccgaaatgactgctaccgagggagccattgtccaaatcaactgcacctatcagactagcggcttcaatggactcttctggtaccaacagcatgcgggcgaagcacctaccttcttgtcctataatgtcttggatggtctcgaagagaaaggcagattctccagtttcctcagccggagcaagggatactcatatcttctcctgaaagagcttcagatgaaggattctgcatcctatctctgtgcttcagtcgatggcaataaccgactcgcctttggaaaagggaatcaagtggtcgtcataccgaatattcagaaccccgaaccagccgtatatcagttgaaggacccaagatctcaggatagtacactctgtttgtttacggactttgactcacaaatcaacgtcccgaagactatggaaagtggtacgttcatcacagataagacggttctggacatgaaggctatggactcaaagagcaacggggcaattgcttggtccaaccagacaagctttacctgtcaggacatttttaaggagactaatgctacttatccctccagcgacgttccgtgtgatgcgactcttaccgagaagtcttttgagaccgatatgaatctcaacttccagaatctgctggtgatcgttctgcggatcctgcttctgaaggttgcaggattcaatcttcttatgactctccggctctggtcttcatgataagaattctgcagtcgacggtaccgcgggcccgggatccgataaaataaaagattttatttagtctccagaaaaaggggggaatgaaagaccccacctgtaggtttggcaagctagcttaagtaacgccattttgcaaggcatggaaaatacataactgagaatagagaagttcagatcaaggttaggaacagagagacagcagaatatgggccaaacaggatatctgtggtaagcagttcctgccccggctcagggccaagaacagatggtccccagatgcggtcccgccctcagcagtttctagagaaccatcagatgtttccagggtgccccaaggacctgaaaatgaccctgtgccttatttgaactaaccaatcagttcgcttctcgcttctgttcgcgcgcttctgctccccgagctcaataaaagagcccacaacccctcactcggcgcgccagtcctccgatagactgcgtcgcccgggtacccgtgtatccaataaaccctcttgcagttgcatccgacttgtggtctcgctgttccttgggagggtctcctctgagtgattgactacccgtcagcgggggtctttcatgggtaacagtttcttgaagttggagaacaacattctgagggtaggagtcgaatattaagtaatcctgactcaattagccactgttttgaatccacatactccaatactcctgaaatccatcgatggagttcattatggacagcgcagaaagagctggggagaattgtgaaattgttatccgctcacaattccacacaacatacgagccggaagcataaagtgtaaagcctggggtgcctaatgagtgagctaactcacattaattgcgttgcgctcactgcccgctttccagtcgggaaacctgtcgtgccagctgcattaatgaatcggccaacgcgcggggagaggcggtttgcgtattgggcgctcttccgcttcctcgctcactgactcgctgcgctcggtcgttcggctgcggcgagcggtatcagctcactcaaaggcggtaatacggttatccacagaatcaggggataacgcaggaaagaacatgtgagcaaaaggccagcaaaaggccaggaaccgtaaaaaggccgcgttgctggcgtttttccataggctccgcccccctgacgagcatcacaaaaatcgacgctcaagtcagaggtggcgaaacccgacaggactataaagataccaggcgtttccccctggaagctccctcgtgcgctctcctgttccgaccctgccgcttaccggatacctgtccgcctttctcccttcgggaagcgtggcgctttctcatagctcacgctgtaggtatctcagttcggtgtaggtcgttcgctccaagctgggctgtgtgcacgaaccccccgttcagcccgaccgctgcgccttatccggtaactatcgtcttgagtccaacccggtaagacacgacttatcgccactggcagcagccactggtaacaggattagcagagcgaggtatgtaggcggtgctacagagttcttgaagtggtggcctaactacggctacactagaagaacagtatttggtatctgcgctctgctgaagccagttaccttcggaaaaagagttggtagctcttgatccggcaaacaaaccaccgctggtagcggtggtttttttgtttgcaagcagcagattacgcgcagaaaaaaaggatctcaagaagatcctttgatcttttctacggggtctgacgctcagtggaacgaaaactcacgttaagggattttggtcatgagattatcaaaaaggatcttcacctagatccttttaaattaaaaatgaagttttaaatcaatctaaagtatatatgagtaaacttggtctgacagttaccaatgcttaatcagtgaggcacctatctcagcgatctgtctatttcgttcatccatagttgcctgactccccgtcgtgtagataactacgatacgggagggcttaccatctggccccagtgctgcaatgataccgcgagacccacgctcaccggctccagatttatcagcaataaaccagccagccggaagggccgagcgcagaagtggtcctgcaactttatccgcctccatccagtctattaattgttgccgggaagctagagtaagtagttcgccagttaatagtttgcgcaacgttgttgccattgctacaggcatcgtggtgtcacgctcgtcgtttggtatggcttcattcagctccggttcccaacgatcaaggcgagttacatgatcccccatgttgtgcaaaaaagcggttagctccttcggtcctccgatcgttgtcagaagtaagttggccgcagtgttatcactcatggttatggcagcactgcataattctcttactgtcatgccatccgtaagatgcttttctgtgactggtgagtactcaaccaagtcattctgagaatagtgtatgcggcgaccgagttgctcttgcccggcgtcaatacgggataataccgcgccacatagcagaactttaaaagtgctcatcattggaaaacgttcttcggggcgaaaactctcaaggatcttaccgctgttgagatccagttcgatgtaacccactcgtgcacccaactgatcttcagcatcttttactttcaccagcgtttctgggtgagcaaaaacaggaaggcaaaatgccgcaaaaaagggaataagggcgacacggaaatgttgaatactcatactcttcctttttcaatattattgaagcatttatcagggttattgtctcatgagcggatacatatttgaatgtatttagaaaaataaacaaataggggttccgcgcacatttccccgaaaagtgccacctgacgtctaagaaaccattattatcatgacattaacctataaaaataggcgtatcacgaggccctttcgtctcgcgcgtttcggtgatgacggtgaaaacctctgacacatgcagctcccggagacggtcacagcttgtctgtaagcggatgccgggagcagacaagcccgtcagggcgcgtcagcgggtgttggcgggtgtcggggctggcttaactatgcggcatcagagcagattgtactgagagtgcaccatatgcggtgtgaaataccgcacagatgcgtaaggagaaaataccgcatcaggcgccattcgccattcaggctgcgcaactgttgggaagggcgatcggtgcgggcctcttcgctattacgccagctggcgaaagggggatgtgctgcaaggcgattaagttgggtaacgccagggttttcccagtcacgacgttgtaaaacgacggcgcaaggaatggtgcatgcaaggagatggcgcccaacagtcccccggccacggggcctgccaccatacccacgccgaaacaagcgctcatgagcccgaagtggcgagcccgatcttccccatcggtgatgtcggcgatataggcgccagcaaccgcacctgtggcgccggtgatgccggccacgatgcgtccggcgtagaggcgattagtccaatttgttaaagacaggatatcagtggtccaggctctagttttgactcaacaatatcaccagctgaagcctatagagtacgagccatagataaaataaaagattttatttagtctccagaaaaaggggggaatgaaagaccccacctgtaggtttggcaagctagcttaagtaacgccattttgcaaggcatggaaaatacataactgagaatagagaagttcagatcaaggttaggaacagagagacagcagaatatgggccaaacaggatatctgtggtaagcagttcctgccccggctcagggccaagaacagatggtccccagatgcggtcccgccctcagcagtttctagagaaccatcagatgtttccagggtgccccaaggacctgaaatgaccctgtgccttatttgaactaaccaatcagttcgcttctcgcttctgttcgcgcgcttctgctccccgagctcaataaaagagcccacaacccctcactcggcgcgccagtcctccgatagactgcgtcgcccgggtacccgtattcccaataaagcctcttgctgtttgcatccgaatcgtggactcgctgatccttgggagggtctcctcagattgattgactgcccacctcgggggtctttcatttggaggttccaccgagatttggagacccctgcccagggaccaccgacccccccgccgggaggtaagctggccagcggtcgtttcgtgtctgtctctgtctttgtgcgtgtttgtgccggcatctaatgtttgcgcctgcgtctgtactagttagctaactagctctgtatctggcggacccgtggtggaactgacgagttcggaacacccggccgcaaccctgggagacgtcccagggacttcgggggccgtttttgtggcccgacctgagtcctaaaatcccgatcgtttaggactctttggtgcaccccccttagaggagggatatgtggttctggtaggagacgagaacctaaaacagttcccgcctccgtctgaatttttgctttcggtttgggaccgaagccgcgccgcgcgtcttgtctgctgcagcatcgttctgtgttgtctctgtctgactgtgtttctgtatttgtctgaaaatatgggcccgggctagcctgttaccactcccttaagtttgaccttaggtcactggaaagatgtcgagcggatcgctcacaaccagtcggtagatgtcaagaagagacgttgggttaccttctgctctgcagaatggccaacctttaacgtcggatggccgcgagacggcacctttaaccgagacctcatcacccaggttaagatcaaggtcttttcacctggcccgcatggacacccagaccaggtcccctacatcgtgacctgggaagccttggcttttgacccccctccctgggtcaagccctttgtacaccctaagcctccgcctcctcttcctccatccgccccgtctctcccccttgaacctcctcgttcgaccccgcctcgatcctccctttatccagccctcactccttctctaggcgcccccatatggccatatgagatcttatatggggcacccccgccccttgtaaacttccctgaccctgacatgacaagagttactaacagcccctctctccaagctcacttacaggctctctacttagtccagcacgaagtctggagacctctggcggcagcctaccaagaacaactggaccgaccggtggtacctcacccttaccgagtcggcgacacagtgtgggtccgccgacaccagactaagaacctagaacctcgctggaaaggaccttacacagtcctgctgaccacccccaccgccctcaaagtagacggcatcgcagcttggatacacgccgcccacgtgaaggctgccgaccccgggggtggaccatcctctagaccg

SEQ ID NO: 38 - DNA, 7310 bp, Artificial Sequence
  Synthetic
ccatggccccggggcttttgtgttgggccttgctttgtttgcttggggcaggcttggtggatgctggagtcacacagtcacccacacacctcattaaaaccaggggacaacaagtcactctgcgctgcagtcctaagtcaggccatgacacagtttcctggtatcaacaggctctggggcagggccctcagttcattttccaatattacgaggaagaggaacgccaacgcggtaatttccccgatcggttctctgggcaccagttcccaaactactcaagtgagttgaacgtaaatgctctcctcctcggagactccgccctctacttgtgtgccagttctcttggttggcggggcggccgatacaatgaacaattttttggacctggtactcggctgaccgtgctagaggacctgcgcaacgtcaccccaccaaaggtcagtttgtttgagccatcaaaggcggagatcgccaacaaacagaaagctacgctcgtgtgtttggctcggggcttcttcccagaccacgtagaactttcctggtgggtcaatggaaaggaggttcattccggagtgtgcactgatccccaagcgtacaaggaatccaactatagctactgtctctcatctcggctccgggtgagtgcgacattctggcataatcctcggaaccactttcgatgccaagtgcagtttcatgggttgagcgaggaagacaagtggcccgagggcagtcctaaaccagtcactcaaaacataagcgccgaggcatggggtagagccgattgtgggattactagcgcttcataccaacaaggggtattgagcgctacaattctttacgaaattctcctcggcaaggcgacgctctacgccgtactggtgtctactctcgtggttatggcaatggtgaaacggaaaaacagcagagccaaaagaagtggttctggcgcgacgaattttagtttgcttaagcaagccggagatgtggaggaaaatcctggaccgatgtggggtgtcttccttttgtacgtcagcatgaagatgggaggcactactgggcaaaacatagatcagcctaccgaaatgactgctaccgagggagccattgtccaaatcaactgcacctatcagactagcggcttcaatggactcttctggtaccaacagcatgcgggcgaagcacctaccttcttgtcctataatgtcttggatggtctcgaagagaaaggcagattctccagtttcctcagccggagcaagggatactcatatcttctcctgaaagagcttcagatgaaggattctgcatcctatctctgtgcttcagtcgatggcaataaccgactcgcctttggaaaagggaatcaagtggtcgtcataccgaatattcagaaccccgaaccagccgtatatcagttgaaggacccaagatctcaggatagtacactctgtttgtttacggactttgactcacaaatcaacgtcccgaagactatggaaagtggtacgttcatcacagataagtgcgttctggacatgaaggctatggactcaaagagcaacggggcaattgcttggtccaaccagacaagctttacctgtcaggacatttttaaggagactaatgctacttatccctccagcgacgttccgtgtgatgcgactcttaccgagaagtcttttgagaccgatatgaatctcaacttccagaatctgctggtgatcgttctgcggatcctgcttctgaaggttgcaggattcaatcttcttatgactctccggctctggtcttcatgataagaattctgcagtcgacggtaccgcgggcccgggatccgataaaataaaagattttatttagtctccagaaaaaggggggaatgaaagaccccacctgtaggtttggcaagctagcttaagtaacgccattttgcaaggcatggaaaatacataactgagaatagagaagttcagatcaaggttaggaacagagagacagcagaatatgggccaaacaggatatctgtggtaagcagttcctgccccggctcagggccaagaacagatggtccccagatgcggtcccgccctcagcagtttctagagaaccatcagatgtttccagggtgccccaaggacctgaaaatgaccctgtgccttatttgaactaaccaatcagttcgcttctcgcttctgttcgcgcgcttctgctccccgagctcaataaaagagcccacaacccctcactcggcgcgccagtcctccgatagactgcgtcgcccgggtacccgtgtatccaataaaccctcttgcagttgcatccgacttgtggtctcgctgttccttgggagggtctcctctgagtgattgactacccgtcagcgggggtctttcatgggtaacagtttcttgaagttggagaacaacattctgagggtaggagtcgaatattaagtaatcctgactcaattagccactgttttgaatccacatactccaatactcctgaaatccatcgatggagttcattatggacagcgcagaaagagctggggagaattgtgaaattgttatccgctcacaattccacacaacatacgagccggaagcataaagtgtaaagcctggggtgcctaatgagtgagctaactcacattaattgcgttgcgctcactgcccgctttccagtcgggaaacctgtcgtgccagctgcattaatgaatcggccaacgcgcggggagaggcggtttgcgtattgggcgctcttccgcttcctcgctcactgactcgctgcgctcggtcgttcggctgcggcgagcggtatcagctcactcaaaggcggtaatacggttatccacagaatcaggggataacgcaggaaagaacatgtgagcaaaaggccagcaaaaggccaggaaccgtaaaaaggccgcgttgctggcgtttttccataggctccgcccccctgacgagcatcacaaaaatcgacgctcaagtcagaggtggcgaaacccgacaggactataaagataccaggcgtttccccctggaagctccctcgtgcgctctcctgttccgaccctgccgcttaccggatacctgtccgcctttctcccttcgggaagcgtggcgctttctcatagctcacgctgtaggtatctcagttcggtgtaggtcgttcgctccaagctgggctgtgtgcacgaaccccccgttcagcccgaccgctgcgccttatccggtaactatcgtcttgagtccaacccggtaagacacgacttatcgccactggcagcagccactggtaacaggattagcagagcgaggtatgtaggcggtgctacagagttcttgaagtggtggcctaactacggctacactagaagaacagtatttggtatctgcgctctgctgaagccagttaccttcggaaaaagagttggtagctcttgatccggcaaacaaaccaccgctggtagcggtggtttttttgtttgcaagcagcagattacgcgcagaaaaaaaggatctcaagaagatcctttgatcttttctacggggtctgacgctcagtggaacgaaaactcacgttaagggattttggtcatgagattatcaaaaaggatcttcacctagatccttttaaattaaaaatgaagttttaaatcaatctaaagtatatatgagtaaacttggtctgacagttaccaatgcttaatcagtgaggcacctatctcagcgatctgtctatttcgttcatccatagttgcctgactccccgtcgtgtagataactacgatacgggagggcttaccatctggccccagtgctgcaatgataccgcgagacccacgctcaccggctccagatttatcagcaataaaccagccagccggaagggccgagcgcagaagtggtcctgcaactttatccgcctccatccagtctattaattgttgccgggaagctagagtaagtagttcgccagttaatagtttgcgcaacgttgttgccattgctacaggcatcgtggtgtcacgctcgtcgtttggtatggcttcattcagctccggttcccaacgatcaaggcgagttacatgatcccccatgttgtgcaaaaaagcggttagctccttcggtcctccgatcgttgtcagaagtaagttggccgcagtgttatcactcatggttatggcagcactgcataattctcttactgtcatgccatccgtaagatgcttttctgtgactggtgagtactcaaccaagtcattctgagaatagtgtatgcggcgaccgagttgctcttgcccggcgtcaatacgggataataccgcgccacatagcagaactttaaaagtgctcatcattggaaaacgttcttcggggcgaaaactctcaaggatcttaccgctgttgagatccagttcgatgtaacccactcgtgcacccaactgatcttcagcatcttttactttcaccagcgtttctgggtgagcaaaaacaggaaggcaaaatgccgcaaaaaagggaataagggcgacacggaaatgttgaatactcatactcttcctttttcaatattattgaagcatttatcagggttattgtctcatgagcggatacatatttgaatgtatttagaaaaataaacaaataggggttccgcgcacatttccccgaaaagtgccacctgacgtctaagaaaccattattatcatgacattaacctataaaaataggcgtatcacgaggccctttcgtctcgcgcgtttcggtgatgacggtgaaaacctctgacacatgcagctcccggagacggtcacagcttgtctgtaagcggatgccgggagcagacaagcccgtcagggcgcgtcagcgggtgttggcgggtgtcggggctggcttaactatgcggcatcagagcagattgtactgagagtgcaccatatgcggtgtgaaataccgcacagatgcgtaaggagaaaataccgcatcaggcgccattcgccattcaggctgcgcaactgttgggaagggcgatcggtgcgggcctcttcgctattacgccagctggcgaaagggggatgtgctgcaaggcgattaagttgggtaacgccagggttttcccagtcacgacgttgtaaaacgacggcgcaaggaatggtgcatgcaaggagatggcgcccaacagtcccccggccacggggcctgccaccatacccacgccgaaacaagcgctcatgagcccgaagtggcgagcccgatcttccccatcggtgatgtcggcgatataggcgccagcaaccgcacctgtggcgccggtgatgccggccacgatgcgtccggcgtagaggcgattagtccaatttgttaaagacaggatatcagtggtccaggctctagttttgactcaacaatatcaccagctgaagcctatagagtacgagccatagataaaataaaagattttatttagtctccagaaaaaggggggaatgaaagaccccacctgtaggtttggcaagctagcttaagtaacgccattttgcaaggcatggaaaatacataactgagaatagagaagttcagatcaaggttaggaacagagagacagcagaatatgggccaaacaggatatctgtggtaagcagttcctgccccggctcagggccaagaacagatggtccccagatgcggtcccgccctcagcagtttctagagaaccatcagatgtttccagggtgccccaaggacctgaaatgaccctgtgccttatttgaactaaccaatcagttcgcttctcgcttctgttcgcgcgcttctgctccccgagctcaataaaagagcccacaacccctcactcggcgcgccagtcctccgatagactgcgtcgcccgggtacccgtattcccaataaagcctcttgctgtttgcatccgaatcgtggactcgctgatccttgggagggtctcctcagattgattgactgcccacctcgggggtctttcatttggaggttccaccgagatttggagacccctgcccagggaccaccgacccccccgccgggaggtaagctggccagcggtcgtttcgtgtctgtctctgtctttgtgcgtgtttgtgccggcatctaatgtttgcgcctgcgtctgtactagttagctaactagctctgtatctggcggacccgtggtggaactgacgagttcggaacacccggccgcaaccctgggagacgtcccagggacttcgggggccgtttttgtggcccgacctgagtcctaaaatcccgatcgtttaggactctttggtgcaccccccttagaggagggatatgtggttctggtaggagacgagaacctaaaacagttcccgcctccgtctgaatttttgctttcggtttgggaccgaagccgcgccgcgcgtcttgtctgctgcagcatcgttctgtgttgtctctgtctgactgtgtttctgtatttgtctgaaaatatgggcccgggctagcctgttaccactcccttaagtttgaccttaggtcactggaaagatgtcgagcggatcgctcacaaccagtcggtagatgtcaagaagagacgttgggttaccttctgctctgcagaatggccaacctttaacgtcggatggccgcgagacggcacctttaaccgagacctcatcacccaggttaagatcaaggtcttttcacctggcccgcatggacacccagaccaggtcccctacatcgtgacctgggaagccttggcttttgacccccctccctgggtcaagccctttgtacaccctaagcctccgcctcctcttcctccatccgccccgtctctcccccttgaacctcctcgttcgaccccgcctcgatcctccctttatccagccctcactccttctctaggcgcccccatatggccatatgagatcttatatggggcacccccgccccttgtaaacttccctgaccctgacatgacaagagttactaacagcccctctctccaagctcacttacaggctctctacttagtccagcacgaagtctggagacctctggcggcagcctaccaagaacaactggaccgaccggtggtacctcacccttaccgagtcggcgacacagtgtgggtccgccgacaccagactaagaacctagaacctcgctggaaaggaccttacacagtcctgctgaccacccccaccgccctcaaagtagacggcatcgcagcttggatacacgccgcccacgtgaaggctgccgaccccgggggtggaccatcctctagaccg

SEQ ID NO: 39 - DNA, 1800 bp, Artificial Sequence
  Synthetic
atggccccggggcttttgtgttgggccttgctttgtttgcttggggcaggcttggtggatgctggagtcacacagtcacccacacacctcattaaaaccaggggacaacaagtcactctgcgctgcagtcctaagtcaggccatgacacagtttcctggtatcaacaggctctggggcagggccctcagttcattttccaatattacgaggaagaggaacgccaacgcggtaatttccccgatcggttctctgggcaccagttcccaaactactcaagtgagttgaacgtaaatgctctcctcctcggagactccgccctctacttgtgtgccagttctcttggttggcggggcggccgatacaatgaacaattttttggacctggtactcggctgaccgtgctagaggacctgcgcaacgtcaccccaccaaaggtcagtttgtttgagccatcaaaggcggagatcgccaacaaacagaaagctacgctcgtgtgtttggctcggggcttcttcccagaccacgtagaactttcctggtgggtcaatggaaaggaggttcattccggagtgtccactgatccccaagcgtacaaggaatccaactatagctactgtctctcatctcggctccgggtgagtgcgacattctggcataatcctcggaaccactttcgatgccaagtgcagtttcatgggttgagcgaggaagacaagtggcccgagggcagtcctaaaccagtcactcaaaacataagcgccgaggcatggggtagagccgattgtgggattactagcgcttcataccaacaaggggtattgagcgctacaattctttacgaaattctcctcggcaaggcgacgctctacgccgtactggtgtctactctcgtggttatggcaatggtgaaacggaaaaacagcagagccaaaagaagtggttctggcgcgacgaattttagtttgcttaagcaagccggagatgtggaggaaaatcctggaccgatgtggggtgtcttccttttgtacgtcagcatgaagatgggaggcactactgggcaaaacatagatcagcctaccgaaatgactgctaccgagggagccattgtccaaatcaactgcacctatcagactagcggcttcaatggactcttctggtaccaacagcatgcgggcgaagcacctaccttcttgtcctataatgtcttggatggtctcgaagagaaaggcagattctccagtttcctcagccggagcaagggatactcatatcttctcctgaaagagcttcagatgaaggattctgcatcctatctctgtgcttcagtcgatggcaataaccgactcgcctttggaaaagggaatcaagtggtcgtcataccgaatattcagaaccccgaaccagccgtatatcagttgaaggacccaagatctcaggatagtacactctgtttgtttacggactttgactcacaaatcaacgtcccgaagactatggaaagtggtacgttcatcacagataagacggttctggacatgaaggctatggactcaaagagcaacggggcaattgcttggtccaaccagacaagctttacctgtcaggacatttttaaggagactaatgctacttatccctccagcgacgttccgtgtgatgcgactcttaccgagaagtcttttgagaccgatatgaatctcaacttccagaatctgctggtgatcgttctgcggatcctgcttctgaaggttgcaggattcaatcttcttatgactctccggctctggtcttcatgataa

SEQ ID NO: 40 - DNA, 1800 bp, Artificial Sequence
  Synthetic
atggccccggggcttttgtgttgggccttgctttgtttgcttggggcaggcttggtggatgctggagtcacacagtcacccacacacctcattaaaaccaggggacaacaagtcactctgcgctgcagtcctaagtcaggccatgacacagtttcctggtatcaacaggctctggggcagggccctcagttcattttccaatattacgaggaagaggaacgccaacgcggtaatttccccgatcggttctctgggcaccagttcccaaactactcaagtgagttgaacgtaaatgctctcctcctcggagactccgccctctacttgtgtgccagttctcttggttggcggggcggccgatacaatgaacaattttttggacctggtactcggctgaccgtgctagaggacctgcgcaacgtcaccccaccaaaggtcagtttgtttgagccatcaaaggcggagatcgccaacaaacagaaagctacgctcgtgtgtttggctcggggcttcttcccagaccacgtagaactttcctggtgggtcaatggaaaggaggttcattccggagtgtgcactgatccccaagcgtacaaggaatccaactatagctactgtctctcatctcggctccgggtgagtgcgacattctggcataatcctcggaaccactttcgatgccaagtgcagtttcatgggttgagcgaggaagacaagtggcccgagggcagtcctaaaccagtcactcaaaacataagcgccgaggcatggggtagagccgattgtgggattactagcgcttcataccaacaaggggtattgagcgctacaattctttacgaaattctcctcggcaaggcgacgctctacgccgtactggtgtctactctcgtggttatggcaatggtgaaacggaaaaacagcagagccaaaagaagtggttctggcgcgacgaattttagtttgcttaagcaagccggagatgtggaggaaaatcctggaccgatgtggggtgtcttccttttgtacgtcagcatgaagatgggaggcactactgggcaaaacatagatcagcctaccgaaatgactgctaccgagggagccattgtccaaatcaactgcacctatcagactagcggcttcaatggactcttctggtaccaacagcatgcgggcgaagcacctaccttcttgtcctataatgtcttggatggtctcgaagagaaaggcagattctccagtttcctcagccggagcaagggatactcatatcttctcctgaaagagcttcagatgaaggattctgcatcctatctctgtgcttcagtcgatggcaataaccgactcgcctttggaaaagggaatcaagtggtcgtcataccgaatattcagaaccccgaaccagccgtatatcagttgaaggacccaagatctcaggatagtacactctgtttgtttacggactttgactcacaaatcaacgtcccgaagactatggaaagtggtacgttcatcacagataagtgcgttctggacatgaaggctatggactcaaagagcaacggggcaattgcttggtccaaccagacaagctttacctgtcaggacatttttaaggagactaatgctacttatccctccagcgacgttccgtgtgatgcgactcttaccgagaagtcttttgagaccgatatgaatctcaacttccagaatctgctggtgatcgttctgcggatcctgcttctgaaggttgcaggattcaatcttcttatgactctccggctctggtcttcatgataa